European Patent Application EP 4 778 939 A1, published July 22, 2026. Title: 一种包含特异性结合GPRC5D和CD3的双特异性抗体的药物组合物. Applicant: 江苏恒瑞医药股份有限公司. The sequence listing filed with the application follows.

SEQUENCE LISTING (84 sequences)

SEQ ID NO: 1 - protein, 118 aa, Mus musculus
  REGION 1..118: note = mAb1-VH
EVQLVESGGGLVKPGGSLKLSCAASGFTFSDYGMHWVRQAPEKGLEWVAFISSGSSTIYYADTVKGRFTISRDNAKNTLFLQMTSLRSEDTAIYYCTRLGPNWYFDVWGTGTTVTVSS

SEQ ID NO: 2 - protein, 113 aa, Mus musculus
  REGION 1..113: note = mAb1-VL
DVVMTQTPLSLSVSLGDQASISCRSSQSLVHSNGNTYLYWYLQKPGQSPKLLIYKVSNRFSGVPDRFSGSGSGTDFTLKISRVEAEDLGVYFCSQSTHVPPLTFGAGTKLELK

SEQ ID NO: 3 - protein, 114 aa, Mus musculus
  REGION 1..114: note = mAb24-VH
QVQLQQSDAELVKPGGSVKISCKVSGYTFTDYPIHWMKQRPEQGLEWMGYVFPRDGSTKYNEKFRVKATWTADKSSSTVYMQLNSLTSDDSAVYFCSRELTAYWGQGTTLRVSS

SEQ ID NO: 4 - protein, 112 aa, Mus musculus
  REGION 1..112: note = mAb24-VL
DVVLTQTPLTLSVTIGQPASISCKSSQSLLHSNGKTYLNWLLQRPGQSPRRLIYLVSKLDSGVPDRFAGSGSGTDFTLKITRVEAEDLGVYYCAQGTHFPRTFGGGSKLEIR

SEQ ID NO: 5 - protein, 5 aa, Mus musculus
  REGION 1..5: note = mAb1-HCDR1
DYGMH

SEQ ID NO: 6 - protein, 17 aa, Mus musculus
  REGION 1..17: note = mAb1-HCDR2
FISSGSSTIYYADTVKG

SEQ ID NO: 7 - protein, 9 aa, Mus musculus
  REGION 1..9: note = mAb1-HCDR3
LGPNWYFDV

SEQ ID NO: 8 - protein, 16 aa, Mus musculus
  REGION 1..16: note = mAb1-LCDR1
RSSQSLVHSNGNTYLY

SEQ ID NO: 9 - protein, 7 aa, Mus musculus
  REGION 1..7: note = mAb1-LCDR2
KVSNRFS

SEQ ID NO: 10 - protein, 10 aa, Mus musculus
  REGION 1..10: note = mAb1-LCDR3
SQSTHVPPLT

SEQ ID NO: 11 - protein, 5 aa, Mus musculus
  REGION 1..5: note = mAb24-HCDR1
DYPIH

SEQ ID NO: 12 - protein, 17 aa, Mus musculus
  REGION 1..17: note = mAb24-HCDR2
YVFPRDGSTKYNEKFRV

SEQ ID NO: 13 - protein, 5 aa, Mus musculus
  REGION 1..5: note = mAb24-HCDR3
ELTAY

SEQ ID NO: 14 - protein, 16 aa, Mus musculus
  REGION 1..16: note = mAb24-LCDR1
KSSQSLLHSNGKTYLN

SEQ ID NO: 15 - protein, 7 aa, Mus musculus
  REGION 1..7: note = mAb24-LCDR2
LVSKLDS

SEQ ID NO: 16 - protein, 9 aa, Mus musculus
  REGION 1..9: note = mAb24-LCDR3
AQGTHFPRT

SEQ ID NO: 17 - protein, 118 aa, synthetic construct
  REGION 1..118: note = hu1H1
EVQLVESGGGLVKPGGSLRLSCAASGFTFSDYGMHWVRQAPGKGLEWVAFISSGSSTIYYADTVKGRFTISRDNAKNSLYLQMNSLRAEDTAVYYCTRLGPNWYFDVWGQGTTVTVSS

SEQ ID NO: 18 - protein, 118 aa, synthetic construct
  REGION 1..118: note = hu1H2
EVQLVESGGGLVKPGGSLRLSCAASGFTFSDYGMHWVRQAPGKGLEWVAFISSGSSNIYYADTVKGRFTISRDNAKNSLYLQMNSLRAEDTAVYYCTRLGPNWYFDVWGQGTTVTVSS

SEQ ID NO: 19 - protein, 118 aa, synthetic construct
  REGION 1..118: note = hu1H3
EVQLVESGGGLVKPGGSLRLSCAASGFTFSDYGMHWVRQAPGKGLEWVAFISSGSSTQYYADTVKGRFTISRDNAKNSLYLQMNSLRAEDTAVYYCTRLGPNWYFDVWGQGTTVTVSS

SEQ ID NO: 20 - protein, 113 aa, synthetic construct
  REGION 1..113: note = hu1L1
DIVMTQTPLSLSVTPGQPASISCRSSQSLVHSNGNTYLYWYLQKPGQSPQLLIYKVSNRFSGVPDRFSGSGSGTDFTLKISRVEAEDVGVYYCSQSTHVPPLTFGQGTKLEIK

SEQ ID NO: 21 - protein, 113 aa, synthetic construct
  REGION 1..113: note = hu1L2
DVVMTQTPLSLSVTPGQPASISCRSSQSLVHSNGNTYLYWYLQKPGQSPKLLIYKVSNRFSGVPDRFSGSGSGTDFTLKISRVEAEDVGVYYCSQSTHVPPLTFGQGTKLEIK

SEQ ID NO: 22 - protein, 113 aa, synthetic construct
  REGION 1..113: note = hu1L3
DVVMTQTPLSLSVTPGQPASISCRSSQSLVHSSGNTYLYWYLQKPGQSPKLLIYKVSNRFSGVPDRFSGSGSGTDFTLKISRVEAEDVGVYYCSQSTHVPPLTFGQGTKLEIK

SEQ ID NO: 23 - protein, 113 aa, synthetic construct
  REGION 1..113: note = hu1L4
DVVMTQTPLSLSVTPGQPASISCRSSQSLVHSQGNTYLYWYLQKPGQSPKLLIYKVSNRFSGVPDRFSGSGSGTDFTLKISRVEAEDVGVYYCSQSTHVPPLTFGQGTKLEIK

SEQ ID NO: 24 - protein, 113 aa, synthetic construct
  REGION 1..113: note = hu1L5
DVVMTQTPLSLSVTPGQPASISCRSSQSLVHSTGNTYLYWYLQKPGQSPKLLIYKVSNRFSGVPDRFSGSGSGTDFTLKISRVEAEDVGVYYCSQSTHVPPLTFGQGTKLEIK

SEQ ID NO: 25 - protein, 113 aa, synthetic construct
  REGION 1..113: note = hu1L6
DVVMTQTPLSLSVTPGQPASISCRSSQSLVHSNVNTYLYWYLQKPGQSPKLLIYKVSNRFSGVPDRFSGSGSGTDFTLKISRVEAEDVGVYYCSQSTHVPPLTFGQGTKLEIK

SEQ ID NO: 26 - protein, 16 aa, synthetic construct
  REGION 1..16: note = hu1L3 LCDR1
RSSQSLVHSSGNTYLY

SEQ ID NO: 27 - protein, 16 aa, synthetic construct
  REGION 1..16: note = hu1L4 LCDR1
RSSQSLVHSQGNTYLY

SEQ ID NO: 28 - protein, 16 aa, synthetic construct
  REGION 1..16: note = hu1L5 LCDR1
RSSQSLVHSTGNTYLY

SEQ ID NO: 29 - protein, 16 aa, synthetic construct
  REGION 1..16: note = hu1L6 LCDR1
RSSQSLVHSNVNTYLY

SEQ ID NO: 30 - protein, 17 aa, synthetic construct
  REGION 1..17: note = hu1H2 HCDR2
FISSGSSNIYYADTVKG

SEQ ID NO: 31 - protein, 17 aa, synthetic construct
  REGION 1..17: note = hu1H3 HCDR2
FISSGSSTQYYADTVKG

SEQ ID NO: 32 - protein, 114 aa, synthetic construct
  REGION 1..114: note = hu24H1
EVQLVQSGAEVKKPGASVKVSCKASGYTFTDYPIHWVRQAPGQGLEWMGYVFPRDGSTKYNEKFRVRVTMTADTSTSTVYMELSSLRSEDTAVYYCSRELTAYWGQGTTVTVSS

SEQ ID NO: 33 - protein, 114 aa, synthetic construct
  REGION 1..114: note = hu24H2
EVQLVQSGAEVKKPGASVKVSCKASGYTFTDYPIHWVRQAPGQGLEWMGYVFPRDGSTKYNEKFRVRVTWTADKSTSTVYMELSSLRSEDTAVYYCSRELTAYWGQGTTVTVSS

SEQ ID NO: 34 - protein, 114 aa, synthetic construct
  REGION 1..114: note = hu24H3
EVQLVQSGAEVKKPGASVKVSCKVSGYTFTDYPIHWMRQAPGQGLEWMGYVFPRDGSTKYNEKFRVRVTWTADKSTSTVYMELSSLRSEDTAVYYCSRELTAYWGQGTTVTVSS

SEQ ID NO: 35 - protein, 112 aa, synthetic construct
  REGION 1..112: note = hu24L1
DVVMTQSPLSLPVTLGQPASISCKSSQSLLHSNGKTYLNWFQQRPGQSPRRLIYLVSKLDSGVPDRFSGSGSGTDFTLKISRVEAEDVGVYYCAQGTHFPRTFGGGTKVEIK

SEQ ID NO: 36 - protein, 112 aa, synthetic construct
  REGION 1..112: note = hu24L2
DVVLTQSPLSLPVTLGQPASISCKSSQSLLHSNGKTYLNWLLQRPGQSPRRLIYLVSKLDSGVPDRFSGSGSGTDFTLKISRVEAEDVGVYYCAQGTHFPRTFGGGTKVEIK

SEQ ID NO: 37 - protein, 112 aa, synthetic construct
  REGION 1..112: note = hu24L3
DVVLTQSPLSLPVTLGQPASISCKSSQSLLHSNVKTYLNWLLQRPGQSPRRLIYLVSKLDSGVPDRFSGSGSGTDFTLKISRVEAEDVGVYYCAQGTHFPRTFGGGTKVEIK

SEQ ID NO: 38 - protein, 112 aa, synthetic construct
  REGION 1..112: note = hu24L4
DVVLTQSPLSLPVTLGQPASISCKSSQSLLHSNLKTYLNWLLQRPGQSPRRLIYLVSKLDSGVPDRFSGSGSGTDFTLKISRVEAEDVGVYYCAQGTHFPRTFGGGTKVEIK

SEQ ID NO: 39 - protein, 112 aa, synthetic construct
  REGION 1..112: note = hu24L5
DVVLTQSPLSLPVTLGQPASISCKSSQSLLHSSGKTYLNWLLQRPGQSPRRLIYLVSKLDSGVPDRFSGSGSGTDFTLKISRVEAEDVGVYYCAQGTHFPRTFGGGTKVEIK

SEQ ID NO: 40 - protein, 112 aa, synthetic construct
  REGION 1..112: note = hu24L6
DVVLTQSPLSLPVTLGQPASISCKSSQSLLHSTGKTYLNWLLQRPGQSPRRLIYLVSKLDSGVPDRFSGSGSGTDFTLKISRVEAEDVGVYYCAQGTHFPRTFGGGTKVEIK

SEQ ID NO: 41 - protein, 16 aa, synthetic construct
  REGION 1..16: note = hu24L3 LCDR1
KSSQSLLHSNVKTYLN

SEQ ID NO: 42 - protein, 16 aa, synthetic construct
  REGION 1..16: note = hu24L4 LCDR1
KSSQSLLHSNLKTYLN

SEQ ID NO: 43 - protein, 16 aa, synthetic construct
  REGION 1..16: note = hu24L5 LCDR1
KSSQSLLHSSGKTYLN

SEQ ID NO: 44 - protein, 16 aa, synthetic construct
  REGION 1..16: note = hu24L6 LCDR1
KSSQSLLHSTGKTYLN

SEQ ID NO: 45 - protein, 330 aa, synthetic construct
  REGION 1..330: note = CH
ASTKGPSVFPLAPSSKSTSGGTAALGCLVKDYFPEPVTVSWNSGALTSGVHTFPAVLQSSGLYSLSSVVTVPSSSLGTQTYICNVNHKPSNTKVDKKVEPKSCDKTHTCPPCPAPEAAGGPSVFLFPPKPKDTLMISRTPEVTCVVVDVSHEDPEVKFNWYVDGVEVHNAKTKPREEQYNSTYRVVSVLTVLHQDWLNGKEYKCKVSNKALPAPIEKTISKAKGQPREPQVYTLPPSRDELTKNQVSLTCLVKGFYPSDIAVEWESNGQPENNYKTTPPVLDSDGSFFLYSKLTVDKSRWQQGNVFSCSVMHEALHNHYTQKSLSLSPGK

SEQ ID NO: 46 - protein, 107 aa, synthetic construct [sequence omitted]

SEQ ID NO: 47 - protein, 448 aa, synthetic construct
  CHAIN 1..448: note = Chi-1-HC
EVQLVESGGGLVKPGGSLKLSCAASGFTFSDYGMHWVRQAPEKGLEWVAFISSGSSTIYYADTVKGRFTISRDNAKNTLFLQMTSLRSEDTAIYYCTRLGPNWYFDVWGTGTTVTVSSASTKGPSVFPLAPSSKSTSGGTAALGCLVKDYFPEPVTVSWNSGALTSGVHTFPAVLQSSGLYSLSSVVTVPSSSLGTQTYICNVNHKPSNTKVDKKVEPKSCDKTHTCPPCPAPEAAGGPSVFLFPPKPKDTLMISRTPEVTCVVVDVSHEDPEVKFNWYVDGVEVHNAKTKPREEQYNSTYRVVSVLTVLHQDWLNGKEYKCKVSNKALPAPIEKTISKAKGQPREPQVYTLPPSRDELTKNQVSLTCLVKGFYPSDIAVEWESNGQPENNYKTTPPVLDSDGSFFLYSKLTVDKSRWQQGNVFSCSVMHEALHNHYTQKSLSLSPGK

SEQ ID NO: 48 - protein, 220 aa, synthetic construct
  CHAIN 1..220: note = Chi-1-LC
DVVMTQTPLSLSVSLGDQASISCRSSQSLVHSNGNTYLYWYLQKPGQSPKLLIYKVSNRFSGVPDRFSGSGSGTDFTLKISRVEAEDLGVYFCSQSTHVPPLTFGAGTKLELKRTVAAPSVFIFPPSDEQLKSGTASVVCLLNNFYPREAKVQWKVDNALQSGNSQESVTEQDSKDSTYSLSSTLTLSKADYEKHKVYACEVTHQGLSSPVTKSFNRGEC

SEQ ID NO: 49 - protein, 444 aa, synthetic construct
  CHAIN 1..444: note = Chi-24-HC
QVQLQQSDAELVKPGGSVKISCKVSGYTFTDYPIHWMKQRPEQGLEWMGYVFPRDGSTKYNEKFRVKATWTADKSSSTVYMQLNSLTSDDSAVYFCSRELTAYWGQGTTLRVSSASTKGPSVFPLAPSSKSTSGGTAALGCLVKDYFPEPVTVSWNSGALTSGVHTFPAVLQSSGLYSLSSVVTVPSSSLGTQTYICNVNHKPSNTKVDKKVEPKSCDKTHTCPPCPAPEAAGGPSVFLFPPKPKDTLMISRTPEVTCVVVDVSHEDPEVKFNWYVDGVEVHNAKTKPREEQYNSTYRVVSVLTVLHQDWLNGKEYKCKVSNKALPAPIEKTISKAKGQPREPQVYTLPPSRDELTKNQVSLTCLVKGFYPSDIAVEWESNGQPENNYKTTPPVLDSDGSFFLYSKLTVDKSRWQQGNVFSCSVMHEALHNHYTQKSLSLSPGK

SEQ ID NO: 50 - protein, 219 aa, synthetic construct
  CHAIN 1..219: note = Chi-24-LC
DVVLTQTPLTLSVTIGQPASISCKSSQSLLHSNGKTYLNWLLQRPGQSPRRLIYLVSKLDSGVPDRFAGSGSGTDFTLKITRVEAEDLGVYYCAQGTHFPRTFGGGSKLEIRRTVAAPSVFIFPPSDEQLKSGTASVVCLLNNFYPREAKVQWKVDNALQSGNSQESVTEQDSKDSTYSLSSTLTLSKADYEKHKVYACEVTHQGLSSPVTKSFNRGEC

SEQ ID NO: 51 - protein, 5 aa, synthetic construct
  REGION 1..5: note = S107E-HCDR1
KYAMN

SEQ ID NO: 52 - protein, 19 aa, synthetic construct
  REGION 1..19: note = S107E-HCDR2
RIRSKYNNYATYYADSVKD

SEQ ID NO: 53 - protein, 14 aa, synthetic construct
  REGION 1..14: note = S107E-HCDR3
HGNFGNEYISYWAY

SEQ ID NO: 54 - protein, 14 aa, synthetic construct
  REGION 1..14: note = S107E-LCDR1
GSSTGAVTSGNYPN

SEQ ID NO: 55 - protein, 7 aa, synthetic construct
  REGION 1..7: note = S107E-LCDR2
GTKFLAP

SEQ ID NO: 56 - protein, 9 aa, synthetic construct
  REGION 1..9: note = S107E-LCDR3
VLWYSNRWV

SEQ ID NO: 57 - protein, 125 aa, synthetic construct
  REGION 1..125: note = S107E-VH
EVQLVESGGGLVQPGGSLKLSCAASGFTFNKYAMNWVRQAPGKGLEWVARIRSKYNNYATYYADSVKDRFTISRDDSKNTAYLQMNNLKTEDTAVYYCVRHGNFGNEYISYWAYWGQGTLVTVSS

SEQ ID NO: 58 - protein, 109 aa, synthetic construct
  REGION 1..109: note = S107E-VL
QTVVTQEPSLTVSPGGTVTLTCGSSTGAVTSGNYPNWVQQKPGQAPRGLIGGTKFLAPGTPARFSGSLLGGKAALTLSGVQPEDEAEYYCVLWYSNRWVFGGGTKLTVL

SEQ ID NO: 59 - protein, 449 aa, synthetic construct
  CHAIN 1..449: note = OB(A0B2)-Hole
EVQLVESGGGLVQPGGSLKLSCAASGFTFNKYAMNWVRQAPGKGLEWVARIRSKYNNYATYYADSVKDRFTISRDDSKNTAYLQMNNLKTEDTAVYYCVRHGNFGNEYISYWAYWGQGTLVTVSSSGAPRFLTCPKASVVSVGKDATLSSQIVGNPFPQVSWEKDKQPVTAGVRFRLAQDGDLYRLKILDLQLSDSGQYVSRARNAHGEAFACLGLQVDAEADKTHTCPPCPAPEAAGGPSVFLFPPKPKDTLMISRTPEVTCVVVDVSHEDPEVKFNWYVDGVEVHNAKTKPREEQYNSTYRVVSVLTVLHQDWLNGKEYKCKVSNKALPAPIEKTISKAKGQPREPQVCTLPPSRDELTKNQVSLSCAVKGFYPSDIAVEWESNGQPENNYKTTPPVLDSDGSFFLVSKLTVDKSRWQQGNVFSCSVMHEALHNHYTQKSLSLSPGK

SEQ ID NO: 60 - protein, 207 aa, synthetic construct
  CHAIN 1..207: note = VL-Titin(A0B2)
QTVVTQEPSLTVSPGGTVTLTCGSSTGAVTSGNYPNWVQQKPGQAPRGLIGGTKFLAPGTPARFSGSLLGGKAALTLSGVQPEDEAEYYCVLWYSNRWVFGGGTKLTVLGIPPKIECLPIDISIDEGKVLTVASCFTGEPTPEVTWSTGGRKIHSQEQGRFHIENTDDSTTLTIKDVQKQDGGLYTLTLRNEFGSDSATVNIHIRSI

SEQ ID NO: 61 - protein, 449 aa, synthetic construct
  CHAIN 1..449: note = Ob(A0B2)-Knob
EVQLVESGGGLVQPGGSLKLSCAASGFTFNKYAMNWVRQAPGKGLEWVARIRSKYNNYATYYADSVKDRFTISRDDSKNTAYLQMNNLKTEDTAVYYCVRHGNFGNEYISYWAYWGQGTLVTVSSSGAPRFLTCPKASVVSVGKDATLSSQIVGNPFPQVSWEKDKQPVTAGVRFRLAQDGDLYRLKILDLQLSDSGQYVSRARNAHGEAFACLGLQVDAEADKTHTCPPCPAPEAAGGPSVFLFPPKPKDTLMISRTPEVTCVVVDVSHEDPEVKFNWYVDGVEVHNAKTKPREEQYNSTYRVVSVLTVLHQDWLNGKEYKCKVSNKALPAPIEKTISKAKGQPREPQVYTLPPCRDELTKNQVSLWCLVKGFYPSDIAVEWESNGQPENNYKTTPPVLDSDGSFFLYSKLTVDKSRWQQGNVFSCSVMHEALHNHYTQKSLSLSPGK

SEQ ID NO: 62 - protein, 103 aa, synthetic construct
  REGION 1..103: note = IgG1(CH1)
ASTKGPSVFPLAPSSKSTSGGTAALGCLVKDYFPEPVTVSWNSGALTSGVHTFPAVLQSSGLYSLSSVVTVPSSSLGTQTYICNVNHKPSNTKVDKKVEPKSC

SEQ ID NO: 63 - protein, 227 aa, synthetic construct
  REGION 1..227: note = IgG1Fc(Knob)
DKTHTCPPCPAPEAAGGPSVFLFPPKPKDTLMISRTPEVTCVVVDVSHEDPEVKFNWYVDGVEVHNAKTKPREEQYNSTYRVVSVLTVLHQDWLNGKEYKCKVSNKALPAPIEKTISKAKGQPREPQVYTLPPCRDELTKNQVSLWCLVKGFYPSDIAVEWESNGQPENNYKTTPPVLDSDGSFFLYSKLTVDKSRWQQGNVFSCSVMHEALHNHYTQKSLSLSPGK

SEQ ID NO: 64 - protein, 227 aa, synthetic construct
  REGION 1..227: note = IgG1Fc(Hole)
DKTHTCPPCPAPEAAGGPSVFLFPPKPKDTLMISRTPEVTCVVVDVSHEDPEVKFNWYVDGVEVHNAKTKPREEQYNSTYRVVSVLTVLHQDWLNGKEYKCKVSNKALPAPIEKTISKAKGQPREPQVCTLPPSRDELTKNQVSLSCAVKGFYPSDIAVEWESNGQPENNYKTTPPVLDSDGSFFLVSKLTVDKSRWQQGNVFSCSVMHEALHNHYTQKSLSLSPGK

SEQ ID NO: 65 - protein, 448 aa, synthetic construct
  CHAIN 1..448: note = F2-0G4S-1-C1
EVQLVESGGGLVKPGGSLRLSCAASGFTFSDYGMHWVRQAPGKGLEWVAFISSGSSTQYYADTVKGRFTISRDNAKNSLYLQMNSLRAEDTAVYYCTRLGPNWYFDVWGQGTTVTVSSASTKGPSVFPLAPSSKSTSGGTAALGCLVKDYFPEPVTVSWNSGALTSGVHTFPAVLQSSGLYSLSSVVTVPSSSLGTQTYICNVNHKPSNTKVDKKVEPKSCDKTHTCPPCPAPEAAGGPSVFLFPPKPKDTLMISRTPEVTCVVVDVSHEDPEVKFNWYVDGVEVHNAKTKPREEQYNSTYRVVSVLTVLHQDWLNGKEYKCKVSNKALPAPIEKTISKAKGQPREPQVYTLPPCRDELTKNQVSLWCLVKGFYPSDIAVEWESNGQPENNYKTTPPVLDSDGSFFLYSKLTVDKSRWQQGNVFSCSVMHEALHNHYTQKSLSLSPGK

SEQ ID NO: 66 - protein, 220 aa, synthetic construct
  CHAIN 1..220: note = F2-0G4S-1-C2
DVVMTQTPLSLSVTPGQPASISCRSSQSLVHSQGNTYLYWYLQKPGQSPKLLIYKVSNRFSGVPDRFSGSGSGTDFTLKISRVEAEDVGVYYCSQSTHVPPLTFGQGTKLEIKRTVAAPSVFIFPPSDEQLKSGTASVVCLLNNFYPREAKVQWKVDNALQSGNSQESVTEQDSKDSTYSLSSTLTLSKADYEKHKVYACEVTHQGLSSPVTKSFNRGEC

SEQ ID NO: 67 - protein, 444 aa, synthetic construct
  CHAIN 1..444: note = F4-0G4S-1-C3
EVQLVQSGAEVKKPGASVKVSCKVSGYTFTDYPIHWMRQAPGQGLEWMGYVFPRDGSTKYNEKFRVRVTWTADKSTSTVYMELSSLRSEDTAVYYCSRELTAYWGQGTTVTVSSASTKGPSVFPLAPSSKSTSGGTAALGCLVKDYFPEPVTVSWNSGALTSGVHTFPAVLQSSGLYSLSSVVTVPSSSLGTQTYICNVNHKPSNTKVDKKVEPKSCDKTHTCPPCPAPEAAGGPSVFLFPPKPKDTLMISRTPEVTCVVVDVSHEDPEVKFNWYVDGVEVHNAKTKPREEQYNSTYRVVSVLTVLHQDWLNGKEYKCKVSNKALPAPIEKTISKAKGQPREPQVCTLPPSRDELTKNQVSLSCAVKGFYPSDIAVEWESNGQPENNYKTTPPVLDSDGSFFLVSKLTVDKSRWQQGNVFSCSVMHEALHNHYTQKSLSLSPGK

SEQ ID NO: 68 - protein, 219 aa, synthetic construct
  CHAIN 1..219: note = F4-0G4S-1-C4
DVVLTQSPLSLPVTLGQPASISCKSSQSLLHSSGKTYLNWLLQRPGQSPRRLIYLVSKLDSGVPDRFSGSGSGTDFTLKISRVEAEDVGVYYCAQGTHFPRTFGGGTKVEIKRTVAAPSVFIFPPSDEQLKSGTASVVCLLNNFYPREAKVQWKVDNALQSGNSQESVTEQDSKDSTYSLSSTLTLSKADYEKHKVYACEVTHQGLSSPVTKSFNRGEC

SEQ ID NO: 69 - protein, 445 aa, synthetic construct
  CHAIN 1..445: note = anti-GPRC5D-HC
QVQLVQSGAEVKKPGASVKVSCKASGYSFTGYTMNWVRQAPGQGLEWMGLINPYNSDTNYAQKLQGRVTMTTDTSTSTAYMELRSLRSDDTAVYYCARVALRVALDYWGQGTLVTVSSASTKGPSVFPLAPCSRSTSESTAALGCLVKDYFPEPVTVSWNSGALTSGVHTFPAVLQSSGLYSLSSVVTVPSSSLGTKTYTCNVDHKPSNTKVDKRVESKYGPPCPPCPAPEAAGGPSVFLFPPKPKDTLMISRTPEVTCVVVDVSQEDPEVQFNWYVDGVEVHNAKTKPREEQFNSTYRVVSVLTVLHQDWLNGKEYKCKVSNKGLPSSIEKTISKAKGQPREPQVYTLPPSQEEMTKNQVSLTCLVKGFYPSDIAVEWESNGQPENNYKTTPPVLDSDGSFFLYSRLTVDKSRWQEGNVFSCSVMHEALHNHYTQKSLSLSLGK

SEQ ID NO: 70 - protein, 214 aa, synthetic construct
  CHAIN 1..214: note = anti-GPRC5D-LC
DIQMTQSPSSLSASVGDRVTITCKASQNVATHVGWYQQKPGKAPKRLIYSASYRYSGVPSRFSGSGSGTEFTLTISNLQPEDFATYYCQQYNRYPYTFGQGTKLEIKRTVAAPSVFIFPPSDEQLKSGTASVVCLLNNFYPREAKVQWKVDNALQSGNSQESVTEQDSKDSTYSLSSTLTLSKADYEKHKVYACEVTHQGLSSPVTKSFNRGEC

SEQ ID NO: 71 - protein, 452 aa, synthetic construct
  CHAIN 1..452: note = anti-CD3E-HC
EVQLVESGGGLVQPGGSLRLSCAASGFTFNTYAMNWVRQAPGKGLEWVARIRSKYNNYATYYAASVKGRFTISRDDSKNSLYLQMNSLKTEDTAVYYCARHGNFGNSYVSWFAYWGQGTLVTVSSASTKGPSVFPLAPCSRSTSESTAALGCLVKDYFPEPVTVSWNSGALTSGVHTFPAVLQSSGLYSLSSVVTVPSSSLGTKTYTCNVDHKPSNTKVDKRVESKYGPPCPPCPAPEAAGGPSVFLFPPKPKDTLMISRTPEVTCVVVDVSQEDPEVQFNWYVDGVEVHNAKTKPREEQFNSTYRVVSVLTVLHQDWLNGKEYKCKVSNKGLPSSIEKTISKAKGQPREPQVYTLPPSQEEMTKNQVSLTCLVKGFYPSDIAVEWESNGQPENNYKTTPPVLDSDGSFLLYSKLTVDKSRWQEGNVFSCSVMHEALHNHYTQKSLSLSLGK

SEQ ID NO: 72 - protein, 215 aa, synthetic construct
  CHAIN 1..215: note = anti-CD3E-LC
QTVVTQEPSLTVSPGGTVTLTCRSSTGAVTTSNYANWVQQKPGQAPRGLIGGTNKRAPGTPARFSGSLLGGKAALTLSGVQPEDEAEYYCALWYSNLWVFGGGTKLTVLGQPKAAPSVTLFPPSSEELQANKATLVCLISDFYPGAVTVAWKADSSPVKAGVETTTPSKQSNNKYAASSYLSLTPEQWKSHRSYSCQVTHEGSTVEKTVAPTECS

SEQ ID NO: 73 - protein, 118 aa, synthetic construct
  REGION 1..118: note = JNJ-64407564-GPRC5D-VH
QVQLVQSGAEVKKPGASVKVSCKASGYSFTGYTMNWVRQAPGQGLEWMGLINPYNSDTNYAQKLQGRVTMTTDTSTSTAYMELRSLRSDDTAVYYCARVALRVALDYWGQGTLVTVSS

SEQ ID NO: 74 - protein, 107 aa, synthetic construct
  REGION 1..107: note = JNJ-64407564-GPRC5D-VL
DIQMTQSPSSLSASVGDRVTITCKASQNVATHVGWYQQKPGKAPKRLIYSASYRYSGVPSRFSGSGSGTEFTLTISNLQPEDFATYYCQQYNRYPYTFGQGTKLEIK

SEQ ID NO: 75 - protein, 448 aa, synthetic construct
  CHAIN 1..448: note = JNJ7564-huIgG1-HC
QVQLVQSGAEVKKPGASVKVSCKASGYSFTGYTMNWVRQAPGQGLEWMGLINPYNSDTNYAQKLQGRVTMTTDTSTSTAYMELRSLRSDDTAVYYCARVALRVALDYWGQGTLVTVSSASTKGPSVFPLAPSSKSTSGGTAALGCLVKDYFPEPVTVSWNSGALTSGVHTFPAVLQSSGLYSLSSVVTVPSSSLGTQTYICNVNHKPSNTKVDKKVEPKSCDKTHTCPPCPAPEAAGGPSVFLFPPKPKDTLMISRTPEVTCVVVDVSHEDPEVKFNWYVDGVEVHNAKTKPREEQYNSTYRVVSVLTVLHQDWLNGKEYKCKVSNKALPAPIEKTISKAKGQPREPQVYTLPPSRDELTKNQVSLTCLVKGFYPSDIAVEWESNGQPENNYKTTPPVLDSDGSFFLYSKLTVDKSRWQQGNVFSCSVMHEALHNHYTQKSLSLSPGK

SEQ ID NO: 76 - protein, 214 aa, synthetic construct; identical to SEQ ID NO: 70
  CHAIN 1..214: note = JNJ7564-huIgG1-LC

SEQ ID NO: 77 - protein, 27 aa, Homo sapiens
  REGION 1..27: note = N
MYKDCIESTGDYFLLCDAEGPWGIILE

SEQ ID NO: 78 - protein, 10 aa, Homo sapiens
  REGION 1..10: note = E2
NQQTAPVRYC

SEQ ID NO: 79 - protein, 23 aa, Homo sapiens
  REGION 1..23: note = E3
TEYVTLIMTRGMMFVNMTPCQLN

SEQ ID NO: 80 - protein, 15 aa, Homo sapiens
  REGION 1..15: note = E4
RGNPQFQRQPQWDDC

SEQ ID NO: 81 - protein, 355 aa, Homo sapiens
  CHAIN 1..355: note = CCR8
MDYTLDLSVTTVTDYYYPDIFSSPCDAELIQTNGKLLLAVFYCLLFVFSLLGNSLVILVLVVCKKLRSITDVYLLNLALSDLLFVFSFPFQTYYLLDQWVFGTVMCKVVSGFYYIGFYSSMFFITLMSVDRYLAVVHAVYALKVRTIRMGTTLCLAVWLTAIMATIPLLVFYQVASEDGVLQCYSFYNQQTLKWKIFTNFKMNILGLLIPFTIFMFCYIKILHQLKRCQNHNKTKAIRLVLIVVIASLLFWVPFNVVLFLTSLHSMHILDGCSISQQLTYATHVTEIISFTHCCVNPVIYAFVGEKFKKHLSEIFQKSCSQIFNYLGRQMPRESCEKSSSCQQHSSRSSSVDYIL

SEQ ID NO: 82 - protein, 445 aa, Homo sapiens
  CHAIN 1..445: note = GIPR
RAETGSKGQTAGELYQRWERYRRECQETLAAAEPPSGLACNGSFDMYVCWDYAAPNATARASCPWYLPWHHHVAAGFVLRQCGSDGQWGLWRDHTQCENPEKNEAFLDQRLILERLQVMYTVGYSLSLATLLLALLILSLFRRLHCTRNYIHINLFTSFMLRAAAILSRDRLLPRPGPYLGDQALALWNQALAACRTAQIVTQYCVGANYTWLLVEGVYLHSLLVLVGGSEEGHFRYYLLLGWGAPALFVIPWVIVRYLYENTQCWERNEVKAIWWIIRTPILMTILINFLIFIRILGILLSKLRTRQMRCRDYRLRLARSTLTLVPLLGVHEVVFAPVTEEQARGALRFAKLGFEIFLSSFQGFLVSVLYCFINKEVQSEIRRGWHHCRLRRSLGEEQRQLPERAFRALPSGSGPGEVPTSRGLSSGTLPGPGNEASRELESYC

SEQ ID NO: 83 - protein, 97 aa, synthetic construct
  REGION 1..97: note = Obscurin(A0B2)
SGAPRFLTCPKASVVSVGKDATLSSQIVGNPFPQVSWEKDKQPVTAGVRFRLAQDGDLYRLKILDLQLSDSGQYVSRARNAHGEAFACLGLQVDAEA

SEQ ID NO: 84 - protein, 98 aa, synthetic construct
  REGION 1..98: note = Titin(A0B2)
GIPPKIECLPIDISIDEGKVLTVASCFTGEPTPEVTWSTGGRKIHSQEQGRFHIENTDDSTTLTIKDVQKQDGGLYTLTLRNEFGSDSATVNIHIRSI